European Patent Application EP 4 592 392 A1, published July 30, 2025. Title: 新型的肿瘤检测标志物TAGMe及其应用. Applicant: 上海奕谱生物科技有限公司. The sequence listing filed with the application follows.

SEQUENCE LISTING (16 sequences)

SEQ ID NO: 1 - DNA, 748 bp, Homo sapiens
  source 1..748: mol_type = genomic DNA
cgaacccgaggctcctggtgccctccgggcagagctctgtgcgctcccagcggccggtgatggcgcgccagccagccaggccccgaccgcaagacaaatggtgcggcgcgcgggtctagtcggcggcgcggaggaggcaggaggaggcaggaggaggcgggaggaggcgaaggctacggaagatcagaagaggggtcaagccatcgctcatgccggcctgaatcggccgctgacctggcccttattaagatgctgggggccgattctacacatagtgcagagggaaaggaattatctaggccattgttagctgaccccaaacggccggataattgagatttctcgaacaatttaaatagatttcaaaaatcctttggccgtaaagataaccgtcacaataaagtagatggcaatacgctagcatttggggagacagggcagagaaaggtggaactgagtgggaataaaaaggaaaagggatgattatagtcgttgggttcgttttggggtttttttattttgtttttgttctgtccccgcaagagaagccgagcaggaaagccagactctgactttgatctctgcaaagggacccgaagcgcgaggtctccttacctgctgggtgaaggcggcctgcggggacgacggggacttgctgggggccccgagcgcgctctcgggtttcgaatcgcagggcaggtcttttgcgtcaggctccagaggcgtgtgcgccaggccaaagccctcg

SEQ ID NO: 2 - DNA, 748 bp, Homo sapiens
  source 1..748: mol_type = genomic DNA
cgagggctttggcctggcgcacacgcctctggagcctgacgcaaaagacctgccctgcgattcgaaacccgagagcgcgctcggggcccccagcaagtccccgtcgtccccgcaggccgccttcacccagcaggtaaggagacctcgcgcttcgggtccctttgcagagatcaaagtcagagtctggctttcctgctcggcttctcttgcggggacagaacaaaaacaaaataaaaaaaccccaaaacgaacccaacgactataatcatcccttttcctttttattcccactcagttccacctttctctgccctgtctccccaaatgctagcgtattgccatctactttattgtgacggttatctttacggccaaaggatttttgaaatctatttaaattgttcgagaaatctcaattatccggccgtttggggtcagctaacaatggcctagataattcctttccctctgcactatgtgtagaatcggcccccagcatcttaataagggccaggtcagcggccgattcaggccggcatgagcgatggcttgacccctcttctgatcttccgtagccttcgcctcctcccgcctcctcctgcctcctcctgcctcctccgcgccgccgactagacccgcgcgccgcaccatttgtcttgcggtcggggcctggctggctggcgcgccatcaccggccgctgggagcgcacagagctctgcccggagggcaccaggagcctcgggttcg

SEQ ID NO: 3 - DNA, 748 bp, synthetic construct
  source 1..748: mol_type = other DNA
ygaattygaggtttttggtgtttttygggtagagttttgtgygtttttagyggtyggtgatggygygttagttagttaggtttygatygtaagataaatggtgyggygygygggtttagtyggyggygyggaggaggtaggaggaggtaggaggaggygggaggaggygaaggttayggaagattagaagaggggttaagttatygtttatgtyggtttgaatyggtygttgatttggtttttattaagatgttgggggtygattttatatatagtgtagagggaaaggaattatttaggttattgttagttgattttaaayggtyggataattgagatttttygaataatttaaatagattttaaaaattttttggtygtaaagataatygttataataaagtagatggtaataygttagtatttggggagatagggtagagaaaggtggaattgagtgggaataaaaaggaaaagggatgattatagtygttgggttygttttggggtttttttattttgtttttgttttgttttygtaagagaagtygagtaggaaagttagattttgattttgatttttgtaaagggattygaagygygaggtttttttatttgttgggtgaaggyggtttgyggggaygayggggatttgttgggggtttygagygygttttygggtttygaatygtagggtaggttttttgygttaggttttagaggygtgtgygttaggttaaagttttyg

SEQ ID NO: 4 - DNA, 748 bp, synthetic construct
  source 1..748: mol_type = other DNA
ygagggttttggtttggygtataygtttttggagtttgaygtaaaagatttgttttgygattygaaattygagagygygttyggggtttttagtaagttttygtygttttygtaggtygtttttatttagtaggtaaggagatttygygtttygggtttttttgtagagattaaagttagagtttggtttttttgttyggttttttttgyggggatagaataaaaataaaataaaaaaattttaaaaygaatttaaygattataattatttttttttttttttatttttatttagttttatttttttttgttttgtttttttaaatgttagygtattgttatttattttattgtgayggttatttttayggttaaaggatttttgaaatttatttaaattgttygagaaattttaattattyggtygtttggggttagttaataatggtttagataatttttttttttttgtattatgtgtagaatyggtttttagtattttaataagggttaggttagyggtygatttaggtyggtatgagygatggtttgattttttttttgatttttygtagttttygttttttttygtttttttttgtttttttttgtttttttygygtygtygattagattygygygtygtattatttgttttgyggtyggggtttggttggttggygygttattatyggtygttgggagygtatagagttttgttyggagggtattaggagtttygggttyg

SEQ ID NO: 5 - DNA, 611 bp, Homo sapiens
  source 1..611: mol_type = genomic DNA
cggtcgcccacgaactcgccctgcagggaacggccttagcacaggcagctcgcgcctgccagcagcgccgcggccccggctatcaacacctcctcctccccactgcgaatgccccgatcgtgctccccaaaacccaatacatccacgcccccaaaaaactgggaacccacgcgggtgccttctgtttaccgcagcgctctcactgcaggcgcttgagtaccagatggcgagagttcgcgcgcaggtggagtggggatcctggcgctaggctacccaggagaggaggggaagggcaacccgcggtcccgcctgtggtgcccggctgtgctcatccccacgccccagaccccaaaaggggctggggaggggcacatctggcggacccctcgcgggggaccaagcgggtttagcaggtgcgccgcctggaacccctacgcccaccttccagggagaaaagtgcctctgcttctcgggaagttcccggcttttcagcacccgggacaacagcagcggcacctggggagaggctctccaccccgccccgcgctcgcttccagtcgccagcttcgtgatcttctgcccggactttctctcacccgccgggcgctgcg

SEQ ID NO: 6 - DNA, 611 bp, Homo sapiens
  source 1..611: mol_type = genomic DNA
cgcagcgcccggcgggtgagagaaagtccgggcagaagatcacgaagctggcgactggaagcgagcgcggggcggggtggagagcctctccccaggtgccgctgctgttgtcccgggtgctgaaaagccgggaacttcccgagaagcagaggcacttttctccctggaaggtgggcgtaggggttccaggcggcgcacctgctaaacccgcttggtcccccgcgaggggtccgccagatgtgcccctccccagccccttttggggtctggggcgtggggatgagcacagccgggcaccacaggcgggaccgcgggttgcccttcccctcctctcctgggtagcctagcgccaggatccccactccacctgcgcgcgaactctcgccatctggtactcaagcgcctgcagtgagagcgctgcggtaaacagaaggcacccgcgtgggttcccagttttttgggggcgtggatgtattgggttttggggagcacgatcggggcattcgcagtggggaggaggaggtgttgatagccggggccgcggcgctgctggcaggcgcgagctgcctgtgctaaggccgttccctgcagggcgagttcgtgggcgaccg

SEQ ID NO: 7 - DNA, 611 bp, synthetic construct
  source 1..611: mol_type = other DNA
yggtygtttaygaattygttttgtagggaayggttttagtataggtagttygygtttgttagtagygtygyggtttyggttattaatatttttttttttttattgygaatgtttygatygtgttttttaaaatttaatatatttaygtttttaaaaaattgggaatttaygygggtgttttttgtttatygtagygtttttattgtaggygtttgagtattagatggygagagttygygygtaggtggagtggggattttggygttaggttatttaggagaggaggggaagggtaattygyggtttygtttgtggtgttyggttgtgtttatttttaygttttagattttaaaaggggttggggaggggtatatttggyggatttttygygggggattaagygggtttagtaggtgygtygtttggaatttttaygtttattttttagggagaaaagtgtttttgtttttygggaagttttyggttttttagtattygggataatagtagyggtatttggggagaggttttttatttygtttygygttygtttttagtygttagtttygtgattttttgttyggatttttttttattygtygggygttgyg

SEQ ID NO: 8 - DNA, 611 bp, synthetic construct
  source 1..611: mol_type = other DNA
ygtagygttyggygggtgagagaaagttygggtagaagattaygaagttggygattggaagygagygyggggyggggtggagagtttttttttaggtgtygttgttgttgtttygggtgttgaaaagtygggaatttttygagaagtagaggtatttttttttttggaaggtgggygtaggggttttaggyggygtatttgttaaattygtttggtttttygygaggggttygttagatgtgtttttttttagttttttttggggtttggggygtggggatgagtatagtygggtattataggygggatygygggttgttttttttttttttttttgggtagtttagygttaggatttttattttatttgygygygaattttygttatttggtatttaagygtttgtagtgagagygttgyggtaaatagaaggtattygygtgggtttttagttttttgggggygtggatgtattgggttttggggagtaygatyggggtattygtagtggggaggaggaggtgttgatagtyggggtygyggygttgttggtaggygygagttgtttgtgttaaggtygttttttgtagggygagttygtgggygatyg

SEQ ID NO: 9 - DNA, 27 bp, synthetic construct
  source 1..27: mol_type = other DNA
gaggaggtaggaggaggtaggaggagg

SEQ ID NO: 10 - DNA, 31 bp, synthetic construct
  source 1..31: mol_type = other DNA
aattcctttccctctacactatatataaaat

SEQ ID NO: 11 - DNA, 29 bp, synthetic construct
  source 1..29: mol_type = other DNA
tttaaaaggggttggggaggggtatattt

SEQ ID NO: 12 - DNA, 28 bp, synthetic construct
  source 1..28: mol_type = other DNA
tctccccaaataccrctactattatccc

SEQ ID NO: 13 - DNA, 30 bp, synthetic construct
  source 1..30: mol_type = other DNA
ttatttaggttattgttagttgattttaaa

SEQ ID NO: 14 - DNA, 33 bp, synthetic construct
  source 1..33: mol_type = other DNA
ctttaacctaacrcacacrcctctaaaacctaa

SEQ ID NO: 15 - DNA, 28 bp, synthetic construct
  source 1..28: mol_type = other DNA
ttgtagggaayggttttagtataggtag

SEQ ID NO: 16 - DNA, 31 bp, synthetic construct
  source 1..31: mol_type = other DNA
tacccttcccctcctctcctaaataacctaa